European Patent Application EP 4 364 728 A1, published May 8, 2024. Title: Pharmaceutical composition containing cell-derived natural or artificial nanovesicles loaded with anti-sense oligonucleotide-based drugs. Applicant: PRIMORIS Co.,Ltd. The sequence listing filed with the application follows.

SEQUENCE LISTING (3 sequences)

SEQ ID NO: 1 - DNA, 20 bp, Artificial Sequence
  anti-sense oligonucleotide
catgatgcgttatctgggtc

SEQ ID NO: 2 - DNA, 20 bp, Artificial Sequence
  anti-sense oligonucleotide
ggccactgattgtgccttat

SEQ ID NO: 3 - DNA, 20 bp, Artificial Sequence
  anti-sense oligonucleotide
actggggaagggaagaaaga